European Patent Specification EP 4 015 526 B1, published October 30, 2024. Title: RECOMBINANT INTERLEUKIN-15 ANALOG. Applicant: LETO LABORATORIES CO., LTD. The sequence listing filed with the application follows.

SEQUENCE LISTING (119 sequences)

SEQ ID NO: 1 - protein, 115 aa, Artificial Sequence
MNWVNVISDLKKIEDLIQSMHIDATLYTESDVHPSCKVTAMKCFLLELQVISLESGDASIHDTVENLIILANNSLSSNGNVTESGCKECEELEEKNIKEFLQSFVHIVQMFINTS

SEQ ID NO: 2 - DNA, 345 bp, Artificial Sequence
atgaactgggtgaacgttatcagcgacctgaagaaaatcgaggatctgattcagagcatgcacattgacgcgaccctgtacaccgaaagcgatgtgcacccgagctgcaaggttaccgcgatgaaatgcttcctgctggagctgcaagtgatcagcctggaaagcggtgacgcgagcattcacgataccgttgagaacctgatcattctggcgaacaacagcctgagcagcaacggtaacgtgaccgagagcggctgcaaggaatgcgaggaactggaggaaaagaacatcaaagaattcctgcagagctttgtgcacatcgttcaaatgtttattaacaccagc

SEQ ID NO: 3 - protein, 133 aa, Artificial Sequence
MNWVNVISDLKKIEDLIQSMHIDATLYTESDVHPSCKVTAMKCFLLELQVISLESGDASIHDTVENLIILANNSLSSNANVTESGCKECEELEEKNIKEFLQSFVHIVQMFINTSGSLPETGGSGGSHHHHHH

SEQ ID NO: 4 - protein, 134 aa, Artificial Sequence
MANWVNVISDLKKIEDLIQSMHIDATLYTESDVHPSCKVTAMKCFLLELQVISLESGDASIHDTVENLIILANNSLSSNANVTESGCKECEELEEKNIKEFLQSFVHIVQMFINTSGSLPETGGSGGSHHHHHH

SEQ ID NO: 5 - protein, 133 aa, Artificial Sequence
MNWVNVISDLKKIEDLIQSMHIRGDLYTESDVHPSCKVTAMKCFLLELQVISLESGDASIHDTVENLIILANNSLSSNANVTESGCKECEELEEKNIKEFLQSFVHIVQMFINTSGSLPETGGSGGSHHHHHH

SEQ ID NO: 6 - protein, 134 aa, Artificial Sequence
MSNWVNVISDLKKIEDLIQSVHIRGDLYTESDVHPSCKVTAMKCFLLELQVISLESGDGSIHDTVENLIILAQQSLSSNANVTESGCKECEELEEKNIKEFLQSFVHIVQMFINTSGSLPETGGSGGSHHHHHH

SEQ ID NO: 7 - protein, 134 aa, Artificial Sequence
MSNWVNVISDLKKIEDLIQSVHIRGDLYTESDVHPSCKVTAMKCFLLELQVISLESGDGSIHDTVENLIILAQQSLSSNANVTESGCKECEELSEKNIKEFLQSFVHIVQVFINTSGSLPETGGSGGSHHHHHH

SEQ ID NO: 8 - protein, 134 aa, Artificial Sequence
MSNWVNVISDLRKIRGDIQSVHIDATLYTESDVHPSCRVTAMKCFLLELQVISLESGDASIHDTVENLIILANQSLSSNANVTESGCKECEELEEKNIKEFLQSFVHIVQLFIQTSGSLPETGGSGGSHHHHHH

SEQ ID NO: 9 - protein, 134 aa, Artificial Sequence
MSNWVNVISDLRKIRGDLNAVHVDATLYTESDVHPSCRVTAMKCFLLELQVISLESGDASIHDTVENLIILANQSLSSNANVTESGCKECEELEEKNIKEFLQSFVHIVQLFIQTSGSLPETGGSGGSHHHHHH

SEQ ID NO: 10 - protein, 134 aa, Artificial Sequence
MSNWVNVISDLRKIRGDIQSVHIDATLYTESDVHPSCRVTAMKCFLLELQVISLESGDASIHDTVENLIILANQSLAAQAQLTESGCKECEELEEKNIKEFLQSFVHIVQLFIQTSGSLPETGGSGGSHHHHHH

SEQ ID NO: 11 - protein, 134 aa, Artificial Sequence
MSNWVNVISDLRKIRGDLNAVHVDATLYTESDVHPSCRVTAMKCFLLELQVISLESGDASIHDTVENLIILANQSLAAQAQLTESGCKECEELEEKNIKEFLQSFVHIVQLFIQTSGSLPETGGSGGSHHHHHH

SEQ ID NO: 12 - protein, 134 aa, Artificial Sequence
MSNWVNVISDLRKIRGDIQSVHIDATLYTESDVHPSCRVTAMKCFLLELQLISLDSGDASIHETVEQLILLANQSLAAQAQLTESGCKECEELEEKNIKEFLQSFVHIVQLFIQTSGSLPETGGSGGSHHHHHH

SEQ ID NO: 13 - DNA, 396 bp, Artificial Sequence
atgtgggtgaacgttatcagcgacctgaagaaaatcgaggatctgattcagagcatgcacattcgtggtgacctgtacaccgaaagcgatgtgcacccgagctgcaaggttaccgcgatgaaatgcttcctgctggagctgcaagtgatcagcctggaaagcggtgacgcgagcattcacgataccgttgagaacctgatcattctggcgaacaacagcctgagcagcaacgcgaacgtgaccgagagcggctgcaaggaatgcgaggaactggaggaaaagaacatcaaagaattcctgcagagctttgtgcacatcgttcaaatgtttattaacaccagcggttctctgccggaaaccggtggttctggtggttctcaccaccaccaccaccac

SEQ ID NO: 14 - DNA, 402 bp, Artificial Sequence
atgagcaactgggtgaacgttatcagcgacctgaagaaaatcgaggatctgattcagagcatgcacattgacgcgaccctgtacaccgaaagcgatgtgcacccgagctgcaaggttaccgcgatgaaatgcttcctgctggagctgcaagtgatcagcctggaaagcggtgacgcgagcattcacgataccgttgagaacctgatcattctggcgaacaacagcctgagcagcaacgcgaacgtgaccgagagcggctgcaaggaatgcgaggaactggaggaaaagaacatcaaagaattcctgcagagctttgtgcacatcgttcaaatgtttattaacaccagcggttctctgccggaaaccggtggttctggtggttctcaccaccaccaccaccac

SEQ ID NO: 15 - DNA, 402 bp, Artificial Sequence
atggccaactgggtgaacgttatcagcgacctgaagaaaatcgaggatctgattcagagcatgcacattgacgcgaccctgtacaccgaaagcgatgtgcacccgagctgcaaggttaccgcgatgaaatgcttcctgctggagctgcaagtgatcagcctggaaagcggtgacgcgagcattcacgataccgttgagaacctgatcattctggcgaacaacagcctgagcagcaacgcgaacgtgaccgagagcggctgcaaggaatgcgaggaactggaggaaaagaacatcaaagaattcctgcagagctttgtgcacatcgttcaaatgtttattaacaccagcggttctctgccggaaaccggtggttctggtggttctcaccaccaccaccaccac

SEQ ID NO: 16 - DNA, 402 bp, Artificial Sequence
atgagcaactgggtgaatgtgattagtgatctgaaaaaaattgaagatctgattcagagtgtgcatattagaggtgatctgtatactgaaagtgatgtgcatccaagctgcaaagtgactgccatgaaatgctttctgctggaactgcaagtgattagcctggaaagtggtgatggcagcattcatgatactgtggaaaacctgattattctggcacagcagagcctgagcagcaatgccaatgtgactgaaagtggctgcaaagaatgtgaagaactggaagaaaaaaacattaaagaatttctgcagagctttgtgcatattgtgcaaatgtttattaacactagtggcagcctgcctgaaactggtggcagtggtggcagccatcatcatcatcatcat

SEQ ID NO: 17 - DNA, 402 bp, Artificial Sequence
atgagcaactgggtgaatgtgattagtgatctgaaaaaaattgaagatctgattcagagtgtgcatattagaggtgatctgtatactgaaagtgatgtgcatccaagctgcaaagtgactgccatgaaatgctttctgctggaactgcaagtgattagcctggaaagtggtgatggcagcattcatgatactgtggaaaacctgattattctggcacagcagagcctgagcagcaatgccaatgtgactgaaagtggctgcaaagaatgtgaagaactgagtgaaaaaaacattaaagaatttctgcagagctttgtgcatattgtgcaagtgtttattaacactagtggcagcctgcctgaaactggtggcagtggtggcagccatcatcatcatcatcat

SEQ ID NO: 18 - DNA, 402 bp, Artificial Sequence
atgagcaactgggtgaatgtgattagtgatctgagaaaaattagaggtgatattcagagtgtgcatattgatgccaccctgtatactgaaagtgatgtgcatccaagctgcagagtgactgccatgaaatgctttctgctggaactgcaagtgattagcctggaaagtggtgatgcaagcattcatgatactgtggaaaacctgattattctggccaatcagagcctgagcagcaatgccaatgtgactgaaagtggctgcaaagaatgtgaagaactggaagaaaaaaacattaaagaatttctgcagagctttgtgcatattgtgcagctgtttattcagactagtggcagcctgcctgaaactggtggcagtggtggcagccatcatcatcatcatcat

SEQ ID NO: 19 - DNA, 402 bp, Artificial Sequence
atgagcaactgggtgaatgtgattagtgatctgagaaaaattagaggtgatctgaatgcagtgcatgtggatgccaccctgtatactgaaagtgatgtgcatccaagctgcagagtgactgccatgaaatgctttctgctggaactgcaagtgattagcctggaaagtggtgatgcaagcattcatgatactgtggaaaacctgattattctggccaatcagagcctgagcagcaatgccaatgtgactgaaagtggctgcaaagaatgtgaagaactggaagaaaaaaacattaaagaatttctgcagagctttgtgcatattgtgcagctgtttattcagactagtggcagcctgcctgaaactggtggcagtggtggcagccatcatcatcatcatcat

SEQ ID NO: 20 - DNA, 402 bp, Artificial Sequence
atgagcaactgggtgaatgtgattagtgatctgagaaaaattagaggtgatattcagagtgtgcatattgatgccaccctgtatactgaaagtgatgtgcatccaagctgcagagtgactgccatgaaatgctttctgctggaactgcaagtgattagcctggaaagtggtgatgcaagcattcatgatactgtggaaaacctgattattctggccaatcagagcctggcagcccaagcacagctgactgaaagtggctgcaaagaatgtgaagaactggaagaaaaaaacattaaagaatttctgcagagctttgtgcatattgtgcagctgtttattcagactagtggcagcctgcctgaaactggtggcagtggtggcagccatcatcatcatcatcat

SEQ ID NO: 21 - DNA, 402 bp, Artificial Sequence
atgagcaactgggtgaatgtgattagtgatctgagaaaaattagaggtgatctgaatgcagtgcatgtggatgccaccctgtatactgaaagtgatgtgcatccaagctgcagagtgactgccatgaaatgctttctgctggaactgcaagtgattagcctggaaagtggtgatgcaagcattcatgatactgtggaaaacctgattattctggccaatcagagcctggcagcccaagcacagctgactgaaagtggctgcaaagaatgtgaagaactggaagaaaaaaacattaaagaatttctgcagagctttgtgcatattgtgcagctgtttattcagactagtggcagcctgcctgaaactggtggcagtggtggcagccatcatcatcatcatcat

SEQ ID NO: 22 - DNA, 402 bp, Artificial Sequence
atgagcaactgggtgaatgtgattagtgatctgagaaaaattagaggtgatattcagagtgtgcatattgatgccaccctgtatactgaaagtgatgtgcatccaagctgcagagtgactgccatgaaatgctttctgctggaactgcagctgattagcctggatagtggtgatgcaagcattcatgaaactgtggaacagctgattctgctggccaatcagagcctggcagcccaagcacagctgactgaaagtggctgcaaagaatgtgaagaactggaagaaaaaaacattaaagaatttctgcagagctttgtgcatattgtgcagctgtttattcagactagtggcagcctgcctgaaactggtggcagtggtggcagccatcatcatcatcatcat

SEQ ID NO: 23 - DNA, 43 bp, Artificial Sequence
taagaaggagatatacatatgaactgggtgaacgttatcagcg

SEQ ID NO: 24 - DNA, 58 bp, Artificial Sequence
gtggtggtggtggtgagaaccagaaccagaaccgctggtgttaataaacatttgaacg

SEQ ID NO: 25 - DNA, 48 bp, Artificial Sequence
gtggtggtggtggtgctcgagttagtggtggtggtggtggtgagaacc

SEQ ID NO: 26 - DNA, 43 bp, Artificial Sequence; identical to SEQ ID NO: 23

SEQ ID NO: 27 - DNA, 49 bp, Artificial Sequence
gtggtggtggtggtggtgagaaccgctggtgttaataaacatttgaacg

SEQ ID NO: 28 - DNA, 44 bp, Artificial Sequence
gtggtggtggtggtgctcgagttagtggtggtggtggtggtgag

SEQ ID NO: 29 - DNA, 43 bp, Artificial Sequence; identical to SEQ ID NO: 23

SEQ ID NO: 30 - DNA, 49 bp, Artificial Sequence
acgctttttggtgctagcaagtgggctggtgttaataaacatttgaacg

SEQ ID NO: 31 - DNA, 45 bp, Artificial Sequence
gtggtggtggtggtgctcgagttaacgctttttggtgctagcaag

SEQ ID NO: 32 - DNA, 43 bp, Artificial Sequence; identical to SEQ ID NO: 23

SEQ ID NO: 33 - DNA, 49 bp, Artificial Sequence
cttctttttagcagactttggaaggctggtgttaataaacatttgaacg

SEQ ID NO: 34 - DNA, 49 bp, Artificial Sequence
gtggtggtggtggtgctcgagttacttctttttagcagactttggaagg

SEQ ID NO: 35 - DNA, 43 bp, Artificial Sequence; identical to SEQ ID NO: 23

SEQ ID NO: 36 - DNA, 46 bp, Artificial Sequence
cttcttttttttcttctttttgctggtgttaataaacatttgaacg

SEQ ID NO: 37 - DNA, 50 bp, Artificial Sequence
gtggtggtggtggtgctcgagttacttcttttttttcttctttttgctgg

SEQ ID NO: 38 - DNA, 43 bp, Artificial Sequence; identical to SEQ ID NO: 23

SEQ ID NO: 39 - DNA, 59 bp, Artificial Sequence
attccacaagctgtggagcaccctgtggagcaccgctggtgttaataaacatttgaacg

SEQ ID NO: 40 - DNA, 59 bp, Artificial Sequence
gtggtggtggtggtgctcgagttaatgatggtgtgcagattccacaagctgtggagcac

SEQ ID NO: 41 - DNA, 43 bp, Artificial Sequence; identical to SEQ ID NO: 23

SEQ ID NO: 42 - DNA, 55 bp, Artificial Sequence
tttgtggtgagcgctagatacaaggctaccgctggtgttaataaacatttgaacg

SEQ ID NO: 43 - DNA, 47 bp, Artificial Sequence
gtggtggtggtggtgctcgagttatttgtggtgagcgctagatacaa

SEQ ID NO: 44 - DNA, 43 bp, Artificial Sequence; identical to SEQ ID NO: 23

SEQ ID NO: 45 - DNA, 55 bp, Artificial Sequence
tttgcgacggtggtgttcgataaggctaccgctggtgttaataaacatttgaacg

SEQ ID NO: 46 - DNA, 43 bp, Artificial Sequence
gtggtggtggtggtgctcgagttatttgcgacggtggtgttcg

SEQ ID NO: 47 - DNA, 43 bp, Artificial Sequence; identical to SEQ ID NO: 23

SEQ ID NO: 48 - DNA, 55 bp, Artificial Sequence
ctttttcttacggtgttctacaatgctaccgctggtgttaataaacatttgaacg

SEQ ID NO: 49 - DNA, 50 bp, Artificial Sequence
gtggtggtggtggtgctcgagttactttttcttacggtgttctacaatgc

SEQ ID NO: 50 - DNA, 43 bp, Artificial Sequence; identical to SEQ ID NO: 23

SEQ ID NO: 51 - DNA, 55 bp, Artificial Sequence
acggcgacgaccagtttttggtacgctaccgctggtgttaataaacatttgaacg

SEQ ID NO: 52 - DNA, 43 bp, Artificial Sequence
gtggtggtggtggtgctcgagttaacggcgacgaccagttttt

SEQ ID NO: 53 - DNA, 43 bp, Artificial Sequence; identical to SEQ ID NO: 23

SEQ ID NO: 54 - DNA, 52 bp, Artificial Sequence
ctttttaccgctagcaaccaggctaccgctggtgttaataaacatttgaacg

SEQ ID NO: 55 - DNA, 46 bp, Artificial Sequence
gtggtggtggtggtgctcgagttactttttaccgctagcaaccagg

SEQ ID NO: 56 - DNA, 43 bp, Artificial Sequence; identical to SEQ ID NO: 23

SEQ ID NO: 57 - DNA, 55 bp, Artificial Sequence
atgatggtgaccagatttacgatggctaccgctggtgttaataaacatttgaacg

SEQ ID NO: 58 - DNA, 48 bp, Artificial Sequence
gtggtggtggtggtgctcgagttaatgatggtgaccagatttacgatg

SEQ ID NO: 59 - DNA, 43 bp, Artificial Sequence; identical to SEQ ID NO: 23

SEQ ID NO: 60 - DNA, 55 bp, Artificial Sequence
cttgtgacgaccagtttttggaaggctaccgctggtgttaataaacatttgaacg

SEQ ID NO: 61 - DNA, 46 bp, Artificial Sequence
gtggtggtggtggtgctcgagttacttgtgacgaccagtttttgga

SEQ ID NO: 62 - DNA, 43 bp, Artificial Sequence; identical to SEQ ID NO: 23

SEQ ID NO: 63 - DNA, 49 bp, Artificial Sequence
atggcgacgaccagtcttctttttgctggtgttaataaacatttgaacg

SEQ ID NO: 64 - DNA, 45 bp, Artificial Sequence
gtggtggtggtggtgctcgagttaatggcgacgaccagtcttctt

SEQ ID NO: 65 - DNA, 43 bp, Artificial Sequence; identical to SEQ ID NO: 23

SEQ ID NO: 66 - DNA, 49 bp, Artificial Sequence
cttatgacgaccagaacgtggaaggctggtgttaataaacatttgaacg

SEQ ID NO: 67 - DNA, 46 bp, Artificial Sequence
gtggtggtggtggtgctcgagttacttatgacgaccagaacgtgga

SEQ ID NO: 68 - DNA, 43 bp, Artificial Sequence; identical to SEQ ID NO: 23

SEQ ID NO: 69 - DNA, 49 bp, Artificial Sequence
gtgatgatggtgagtttcaaccaggctggtgttaataaacatttgaacg

SEQ ID NO: 70 - DNA, 48 bp, Artificial Sequence
gtggtggtggtggtgctcgagttagtgatgatggtgagtttcaaccag

SEQ ID NO: 71 - DNA, 43 bp, Artificial Sequence; identical to SEQ ID NO: 23

SEQ ID NO: 72 - DNA, 49 bp, Artificial Sequence
atgatggtgagtttctggacgaacgctggtgttaataaacatttgaacg

SEQ ID NO: 73 - DNA, 47 bp, Artificial Sequence
gtggtggtggtggtgctcgagttaatgatggtgagtttctggacgaa

SEQ ID NO: 74 - DNA, 43 bp, Artificial Sequence; identical to SEQ ID NO: 23

SEQ ID NO: 75 - DNA, 34 bp, Artificial Sequence
cttttttttgctggtgttaataaacatttgaacg

SEQ ID NO: 76 - DNA, 50 bp, Artificial Sequence
gtggtggtggtggtgctcgagttacttttttttgctggtgttaataaaca

SEQ ID NO: 77 - DNA, 43 bp, Artificial Sequence; identical to SEQ ID NO: 23

SEQ ID NO: 78 - DNA, 40 bp, Artificial Sequence
atgatgatggtgacggctggtgttaataaacatttgaacg

SEQ ID NO: 79 - DNA, 44 bp, Artificial Sequence
gtggtggtggtggtgctcgagttaatgatgatggtgacggctgg

SEQ ID NO: 80 - DNA, 43 bp, Artificial Sequence; identical to SEQ ID NO: 23

SEQ ID NO: 81 - DNA, 49 bp, Artificial Sequence
atgatgatggtgagtttcacgcttgctggtgttaataaacatttgaacg

SEQ ID NO: 82 - DNA, 47 bp, Artificial Sequence
gtggtggtggtggtgctcgagttaatgatgatggtgagtttcacgct

SEQ ID NO: 83 - DNA, 43 bp, Artificial Sequence; identical to SEQ ID NO: 23

SEQ ID NO: 84 - DNA, 52 bp, Artificial Sequence
accaccagaaccaccggtttccggcagagaaccgctggtgttaataaacatt

SEQ ID NO: 85 - DNA, 57 bp, Artificial Sequence
gtggtggtggtggtgctcgagttagtggtggtggtggtggtgagaaccaccagaacc

SEQ ID NO: 86 - DNA, 43 bp, Artificial Sequence; identical to SEQ ID NO: 23

SEQ ID NO: 87 - DNA, 49 bp, Artificial Sequence
cttctttttaccagtttcaaggtggctggtgttaataaacatttgaacg

SEQ ID NO: 88 - DNA, 49 bp, Artificial Sequence
gtggtggtggtggtgctcgagttacttctttttaccagtttcaaggtgg

SEQ ID NO: 89 - DNA, 43 bp, Artificial Sequence; identical to SEQ ID NO: 23

SEQ ID NO: 90 - DNA, 49 bp, Artificial Sequence
acggcgacgaccagattcaacatggctggtgttaataaacatttgaacg

SEQ ID NO: 91 - DNA, 43 bp, Artificial Sequence
gtggtggtggtggtgctcgagttaacggcgacgaccagattca

SEQ ID NO: 92 - DNA, 43 bp, Artificial Sequence; identical to SEQ ID NO: 23

SEQ ID NO: 93 - DNA, 49 bp, Artificial Sequence
cttctttttaccagtatgacgacggctggtgttaataaacatttgaacg

SEQ ID NO: 94 - DNA, 49 bp, Artificial Sequence
gtggtggtggtggtgctcgagttacttctttttaccagtatgacgacgg

SEQ ID NO: 95 - DNA, 43 bp, Artificial Sequence; identical to SEQ ID NO: 23

SEQ ID NO: 96 - DNA, 49 bp, Artificial Sequence
atgatggtgaccagtcttaacatggctggtgttaataaacatttgaacg

SEQ ID NO: 97 - DNA, 49 bp, Artificial Sequence
gtggtggtggtggtgctcgagttaatgatggtgaccagtcttaacatgg

SEQ ID NO: 98 - DNA, 43 bp, Artificial Sequence; identical to SEQ ID NO: 23

SEQ ID NO: 99 - DNA, 49 bp, Artificial Sequence
atgatgacgaccagacttaacatggctggtgttaataaacatttgaacg

SEQ ID NO: 100 - DNA, 49 bp, Artificial Sequence
gtggtggtggtggtgctcgagttaatgatgacgaccagacttaacatgg

SEQ ID NO: 101 - DNA, 43 bp, Artificial Sequence; identical to SEQ ID NO: 23

SEQ ID NO: 102 - DNA, 49 bp, Artificial Sequence
gtgacgatggctagacttaacatggctggtgttaataaacatttgaacg

SEQ ID NO: 103 - DNA, 49 bp, Artificial Sequence
gtggtggtggtggtgctcgagttagtgacgatggctagacttaacatgg

SEQ ID NO: 104 - DNA, 43 bp, Artificial Sequence; identical to SEQ ID NO: 23

SEQ ID NO: 105 - DNA, 55 bp, Artificial Sequence
gctaccgctaccgctaccgctaccgctaccgctggtgttaataaacatttgaacg

SEQ ID NO: 106 - DNA, 43 bp, Artificial Sequence
atgatggtgaccagactttaccaggctaccgctaccgctaccg

SEQ ID NO: 107 - DNA, 48 bp, Artificial Sequence
gtggtggtggtggtgctcgagttaatgatggtgaccagactttaccag

SEQ ID NO: 108 - DNA, 43 bp, Artificial Sequence; identical to SEQ ID NO: 23

SEQ ID NO: 109 - DNA, 49 bp, Artificial Sequence
cttatggtgaccgctctttggacggctggtgttaataaacatttgaacg

SEQ ID NO: 110 - DNA, 46 bp, Artificial Sequence
gtggtggtggtggtgctcgagttacttatggtgaccgctctttgga

SEQ ID NO: 111 - DNA, 43 bp, Artificial Sequence; identical to SEQ ID NO: 23

SEQ ID NO: 112 - DNA, 58 bp, Artificial Sequence
gtggtggtggtggtgctcgagttaacactttttgctggtgttaataaacatttgaacg

SEQ ID NO: 113 - DNA, 43 bp, Artificial Sequence; identical to SEQ ID NO: 23

SEQ ID NO: 114 - DNA, 49 bp, Artificial Sequence
atggtgtttaccagccttgtgaaggctggtgttaataaacatttgaacg

SEQ ID NO: 115 - DNA, 47 bp, Artificial Sequence
gtggtggtggtggtgctcgagttaatggtgtttaccagccttgtgaa

SEQ ID NO: 116 - DNA, 43 bp, Artificial Sequence; identical to SEQ ID NO: 23

SEQ ID NO: 117 - DNA, 52 bp, Artificial Sequence
gtggtggtggtggtgctcgagttatttgctggtgttaataaacatttgaacg

SEQ ID NO: 118 - DNA, 43 bp, Artificial Sequence; identical to SEQ ID NO: 23

SEQ ID NO: 119 - DNA, 55 bp, Artificial Sequence
gtggtggtggtggtgctcgagttactttttgctggtgttaataaacatttgaacg